European Patent Application EP 4 563 587 A1, published June 4, 2025. Title: Antibacterial Protein Having Strong Lytic Activity to Staphylococci including Staphylococcus aureus. Applicant: iNtRON Biotechnology, Inc. The sequence listing filed with the application follows.

SEQUENCE LISTING (2 sequences)

SEQ ID NO: 1 - protein, 345 aa, Artificial Sequence
MAKTQAEINKRLDAYAKGTVDSPYRIKKATSYDPSFGVMEAGAIDADGYYHAQCQDLITDYVLWLTDNKVRTWGNAKDQIKQSYGTGFKIHENKPSTVPKKGWIAVFTSGSYQQWGHIGIVYDGGNTSTFTILEQNWNGYANKKPTKRVDNYYGLTHFIEIPVKAGTTVKKETAKKSASKTPAPKKKATLKVSKNHINYTMDKRGKKPEGMVIHNDAGRSSGQQYENSLANAGYARYANGTPATRPVTGSWKKNQYGTWYKPENATFVNGNQPIVTRIGSPFLNAPVGGNLPAGATIVYDEVSIQAGHIWIGYNAYNGNRVYSPVRTCQGVPPNHIPGVAWGVFK

SEQ ID NO: 2 - DNA, 5107 bp, Artificial Sequence
  source 1..5107: mol_type = other DNA
aagaaaccaattgtccatattgcatcagacattgccgtcactgcgtcttttactggctcttctcgctaaccaaaccggtaaccccgcttattaaaagcattctgtaacaaagcgggaccaaagccatgacaaaaacgcgtaacaaaagtgtctataatcacggcagaaaagtccacattgattatttgcacggcgtcacactttgctatgccatagcatttttatccataagattagcggatcctacctgacgctttttatcgcaactctctactgtttctccatacccgtttttttgggctagaaataattttgtttaactttaagaaggagatatacatccccatggccaagacacaagcagagattaataagcggctggatgcatacgccaagggtactgtagactctccctatcgtatcaaaaaggcaactagttacgatcctagttttggagttatggaagctggtgcaatagacgcggacggttattaccacgcccagtgccaggatcttatcaccgattacgttctgtggctgacggacaacaaggtcagaacatggggaaacgctaaagaccaaatcaagcaatcatatgggaccggcttcaaaattcacgaaaacaagccgtccacggtcccaaagaaggggtggatcgctgtgtttacgagtggctcttaccaacaatgggggcacataggaattgtctatgacggaggtaacacatcgacatttaccatcttagaacaaaattggaacggatacgctaataaaaagcccacgaagcgtgtcgataattattacggactgactcacttcattgaaatacctgtcaaagccgggacaacagttaaaaaggagaccgcaaaaaaaagcgcatccaaaacccctgcccctaaaaagaaggctaccttgaaagtgtccaagaaccatataaactatacgatggataagcggggaaaaaaacccgaaggaatggtaattcacaacgatgcaggtcgttcatcaggccagcagtacgaaaactcactggctaacgccggatacgctcgttatgcgaacgggacgccagcgacacgccctgttacggggtcatggaagaagaaccaatacggaacttggtacaaaccagagaacgcaacatttgtcaacggaaatcagccaattgtcactagaatagggtcaccctttcttaacgcgccggtcgggggtaacttacccgctggtgccaccattgtttatgatgaagtctcgattcaggctgggcatatttggataggatacaatgcttataacgggaaccgtgtatatagtcccgttcgtacttgccaaggagtccccccaaaccatattccgggagtcgcttggggtgtctttaagtaagcggccgcaagggcgagcttgaaggtaagcctatccctaaccctctcctcggtctcgattctacgcgtaccggtcatcatcaccatcaccattgagtttaaacggtctccagcttggctgttttggcggatgagagaagattttcagcctgatacagattaaatcagaacgcagaagcggtctgataaaacagaatttgcctggcggcagtagcgcggtggtcccacctgaccccatgccgaactcagaagtgaaacgccgtagcgccgatggtagtgtggggtctccccatgcgagagtagggaactgccaggcatcaaataaaacgaaaggctcagtcgaaagactgggcctttcgttttatctgttgtttgtcggtgaacgctctcctgagtaggacaaatccgccgggagcggatttgaacgttgcgaagcaacggcccggagggtggcgggcaggacgcccgccataaactgccaggcatcaaattaagcagaaggccatcctgacggatggcctttttgcgtttctacaaactcttttgtttatttttctaaatacattcaaatatgtatccgctcatgagattatcaaaaaggatcttcacctagatccttttaaattaaaaatgaagttttaaatcaatctaaagtatatatgagtaaacttggtctgacagttaggcgtcgcttggtcggtcatttcgaaccccagagtcccgctcagaagaactcgtcaagaaggcgatagaaggcgatgcgctgcgaatcgggagcggcgataccgtaaagcacgaggaagcggtcagcccattcgccgccaagctcttcagcaatatcacgggtagccaacgctatgtcctgatagcggtccgccacacccagccggccacagtcgatgaatccagaaaagcggccattttccaccatgatattcggcaagcaggcatcgccatgtgtcacgacgagatcctcgccgtcgggcatgcgcgccttgagcctggcgaacagttcggctggcgcgagcccctgatgctcttcgtccagatcatcctgatcgacaagaccggcttccatccgagtacgtgctcgctcgatgcgatgtttcgcttggtggtcgaatgggcaggtagccggatcaagcgtatgcagccgccgcattgcatcagccatgatggatactttctcggcaggagcaaggtgagatgacaggagatcctgccccggcacttcgcccaatagcagccagtcccttcccgcttcagtgacaacgtcgagcacagctgcgcaaggaacgcccgtcgtggccagccacgatagccgcgctgcctcgtcctgcagttcattcagggcaccggacaggtcggtcttgacaaaaagaaccgggcgcccctgcgctgacagccggaacacggcggcatcagagcagccgattgtcagttgtgcccagtcatagccgaatagcctctccacccaagcggccggagaacctgcgtgcaatccatcttgttcaatcatactcttcctttttcaatattattgaagcatttatcagggttattgtctcatgaccaaaatcccttaacgtgagttttcgttccactgagcgtcagaccccgtagaaaagatcaaaggatcttcttgagatcctttttttctgcgcgtaatctgctgcttgcaaacaaaaaaaccaccgctaccagcggtggtttgtttgccggatcaagagctaccaactctttttccgaaggtaactggcttcagcagagcgcagataccaaatactgtccttctagtgtagccgtagttaggccaccacttcaagaactctgtagcaccgcctacatacctcgctctgctaatcctgttaccagtggctgctgccagtggcgataagtcgtgtcttaccgggttggactcaagacgatagttaccggataaggcgcagcggtcgggctgaacggggggttcgtgcacacagcccagcttggagcgaacgacctacaccgaactgagatacctacagcgtgagctatgagaaagcgccacgcttcccgaagggagaaaggcggacaggtatccggtaagcggcagggtcggaacaggagagcgcacgagggagcttccagggggaaacgcctggtatctttatagtcctgtcgggtttcgccacctctgacttgagcgtcgatttttgtgatgctcgtcaggggggcggagcctatggaaaaacgccagcaacgcggcctttttacggttcctggccttttgctggccttttgctcacatgttctttcctgcgttatcccctgattctgtggataaccgtattaccgcctttgagtgagctgataccgctcgccgcagccgaacgaccgagcgcagcgagtcagtgagcgaggaagcggaagagcgcctgatgcggtattttctccttacgcatctgtgcggtatttcacaccgcatatggtgcactctcagtacaatctgctctgatgccgcatagttaagccagtatacactccgctatcgctacgtgactgggtcatggctgcgccccgacacccgccaacacccgctgacgcgccctgacgggcttgtctgctcccggcatccgcttacagacaagctgtgaccgtctccgggagctgcatgtgtcagaggttttcaccgtcatcaccgaaacgcgcgaggcagcagatcaattcgcgcgcgaaggcgaagcggcatgcataatgtgcctgtcaaatggacgaagcagggattctgcaaaccctatgctactccgtcaagccgtcaattgtctgattcgttaccaattatgacaacttgacggctacatcattcactttttcttcacaaccggcacggaactcgctcgggctggccccggtgcattttttaaatacccgcgagaaatagagttgatcgtcaaaaccaacattgcgaccgacggtggcgataggcatccgggtggtgctcaaaagcagcttcgcctggctgatacgttggtcctcgcgccagcttaagacgctaatccctaactgctggcggaaaagatgtgacagacgcgacggcgacaagcaaacatgctgtgcgacgctggcgatatcaaaattgctgtctgccaggtgatcgctgatgtactgacaagcctcgcgtacccgattatccatcggtggatggagcgactcgttaatcgcttccatgcgccgcagtaacaattgctcaagcagatttatcgccagcagctccgaatagcgcccttccccttgcccggcgttaatgatttgcccaaacaggtcgctgaaatgcggctggtgcgcttcatccgggcgaaagaaccccgtattggcaaatattgacggccagttaagccattcatgccagtaggcgcgcggacgaaagtaaacccactggtgataccattcgcgagcctccggatgacgaccgtagtgatgaatctctcctggcgggaacagcaaaatatcacccggtcggcaaacaaattctcgtccctgatttttcaccaccccctgaccgcgaatggtgagattgagaatataacctttcattcccagcggtcggtcgataaaaaaatcgagataaccgttggcctcaatcggcgttaaacccgccaccagatgggcattaaacgagtatcccggcagcaggggatcattttgcgcttcagccatacttttcatactcccgccattcagag